European Patent Application EP 4 299 594 A1, published January 3, 2024. Title: GUCY2C BINDING POLYPEPTIDE AND USES THEREOF. Applicant: LG CHEM, LTD. The sequence listing filed with the application follows.

SEQUENCE LISTING (115 sequences)

SEQ ID NO: 1 - protein, 246 aa, Artificial Sequence
  Synthetic_GUCY2C-binding scFv
QVQLVQSGAEVKKPGASVKVSCKASGYTFTSYYMHWVRQAPGQGLEWMGIINPSGGSTSYAQEFQGRVTMTRDTSTSTVYMELSSLRSEDTAVYYCARDGQWLQFDYWGQGTLVTVSSGGGGSGGGGSGGGASDIVMTQSPLSLPVTLGQPASISCRSSQSLLKKSDGNTYLSWYHQRPGQSPRRLIYKVSNRDSGVPDRFSGSGSDTDFTLKISRVETEDVGIYYCMQGSHWPPTFGQGTKVEIK

SEQ ID NO: 2 - protein, 243 aa, Artificial Sequence
  Synthetic_GUCY2C-binding scFv
EVQLVQPGAEVKKPGSSVKVSCKASGGTLSSYAISWVRQAPGQGLEWMGRIIPILGITNYAQKFQGRVTITADKSTSTAYMELSSLRSEDTAVYFCARDQRPASMDVWGQGTLVTVSSGGGGSGGGGSGGGASQSELTQPASVSGSPGQSITISCTGTSSDVGGYIYVSWYQQHPGKVPKLMIHDVSHRPSGVSNRFSGSRSGNTASLTISGLQAEDEADYFCSSYAGSNNYVFGTGTKVTVL

SEQ ID NO: 3 - protein, 245 aa, Artificial Sequence
  Synthetic_GUCY2C-binding scFv
QVQLVQSGAEVKKPGSSVKVSCKASGGTFSSYTISWVRQAPGQELEWMGRIIPILGIANYAQKFQGRVTITADKSTSTAYMELSSLRSEDTAVYYCARDYSSSWNSMDVWGQGTLVTVSSGGGGSGGGGSGGGASQSGLTQPPSASGSPGQSVTISCTGTSSDIGYYHYVSWYQQHPGKAPKLMIYEDSKRPSGISNRFSGSKSGTTASLTVSGLQAEDEAHYYCSSFTSRSTWVFGGGTQLTVL

SEQ ID NO: 4 - protein, 243 aa, Artificial Sequence
  Synthetic_GUCY2C-binding scFv
EVQLVQPGAEVKKPGSSVKVSCKASGGTLSSYAISWVRQAPGQGLEWMGRIIPILGITNYAQKFQGRVTITADKSTSTAYMELSSLRSEDTAVYFCARDQRPASMDVWGQGTLVTVSSGGGGSGGGGSGGGASQSELTQPASVSGSPGQSITISCTGTSSDVGGYIYVSWYQQHPGKVPKLMIHDVSHRPSGVSNRFSGSRSGNTASLTISGLQAEDEADYFCSSYTSSNNYYFGTGTKVTVL

SEQ ID NO: 5 - protein, 245 aa, Artificial Sequence
  Synthetic_GUCY2C-binding scFv
QVQLVQSGAEVKKPGSSVKVSCKASGGTFSSYTITWVRQAPGQGLEWMGRIIPVLGIANYAQKFQGRVTITADKSTSTAYMELSSLRSEDTAVYYCARDYSSSWNSMDVWGQGTLVTVSSGGGGSGGGGSGGGASQSGLTQPRSVSGSPGQSVTISCTGTSSDVGGYNYVSWYQQHPGKAPKLMIYDVSKRPSGVPDRFSGSKSGNTASLTVSGLHAEDEADYYCSSYAGSNNFVFGTGTKVTVL

SEQ ID NO: 6 - protein, 245 aa, Artificial Sequence
  Synthetic_GUCY2C-binding scFv
QVQLVQSGAEVKKPGSSVKVSCKASGGTFGSYTISWVRQAPGQGLEWMGRIIPILGIANYAQKFQGRVTITADKSTSTAYMELSSLRSEDTAVYYCARDYSSSWNSMDVWGQGTLVTVSSGGGGSGGGGSGGGASQSGLTQPRSVSGSPGQSVTISCTGTSSDVGAYNYVSWYQQHPGKAPKLMIYEVSKRPSGVPDRFSASKSGNTASLTVSGLQAEDEADYYCSSYAGSNNWVFGGGTKLTVL

SEQ ID NO: 7 - protein, 244 aa, Artificial Sequence
  Synthetic_GUCY2C-binding scFv
QVQLQESGPGLVKPSETLSLTCTVSGGSISSYYWSWIRQPPGKGLEWIGSIYYSGSTNYNPSLKSRVTISRDKSKNQLFLKLNSMTAADTAVYYCARDVWGSGQSFDSWGQGTLVTVSSGGGGSGGGGSGGGASNFMLTQPHSVSESPGKTVTISCTRSSGSIASNYVQWYQQRLGSSPTTVIYEHSRRPSGVPDRFSASIDSSSNSASLTISGLKTEDEADYYCQSYDVSNRVFGGGTKLTVL

SEQ ID NO: 8 - protein, 246 aa, Artificial Sequence
  Synthetic_GUCY2C-binding scFv
EVQLLESGGGLVQPGGSLRLSCAASGFTFSSYWMSWVRQAPGKGLEWVANIKQDGSEKYYVDSVKGRFTISRDNAKNSLYLQMNSLRAEDTAVYYCAKAPWYSSSPTPYGMDVWGQGTLVTVSSGGGGSGGGGSGGGASDIQMTQSPSSLSASVGDRVTITCQASQDISNYLNWYQQKPGKAPRRLIYGASTLMSGVPSRFSGSGSGTDFTLTISSLQPEDFATYYCQQSYSTPLTFGGGTKVEIK

SEQ ID NO: 9 - protein, 246 aa, Artificial Sequence
  Synthetic_GUCY2C-binding scFv
EVQLVQSGAEVKKPGSSVKVSCKASGGTFSSYAISWVRQAPGQGLEWMGGIIPIFGTANYAQKFQGRVTITADESTSTAYMELSSLRSEDTAVYYCARTRYIWGSYRAYGMDVWGQGTMVTVSSGGGGSGGGGSGGGASDIQMTQSPSSMSASVGDRVTITCRASQSISSHLNWYQQLPGNAPTLLIYYASNLQSGVPSRFSGSGSGTDFTLTISSLQPDDFATYYCQQSISLPYTFGQGTKVEIK

SEQ ID NO: 10 - protein, 243 aa, Artificial Sequence
  Synthetic_GUCY2C-binding scFv
EVQLVQPGAEVKKPGSSVKVSCKASGGTLSSYAISWVRQAPGQGLEWMGRIIPILGITNYAQKFQGRVTITADKSTSTAYMELSSLRSEDTAVYFCARDQRPASMDVWGQGTLVTVSSGGGGSGGGGSGGGASQSELTQPASVSGSPGQSITISCTGTSSDVGGYIYVSWYQQHPGKVPKLMIHDVSHRPSGVSNRFSGSRSGNTASLTISGLQAEDEADYFCSSYTSSNNYVFGTGTKVTVL

SEQ ID NO: 11 - protein, 243 aa, Artificial Sequence
  Synthetic_GUCY2C-binding scFv
EVQLVQPGAEVKKPGSSVKVSCKASGGTLSSYAISWVRQAPGQGLEWMGRIIPILGITNYAQKFQGRVTITADKSTSTAYMELSSLRSEDTAVYFCARDQRPASMDVWGQGTLVTVSSGGGGSGGGGSGGGASQSGLTQPASVSGSPGQSITISCTGTSSDVGGYNYVSWYQQHPGKAPKLMIYEVSNRPSGVSNRFSGSKSGNTASLTISGLQAEDEADYYCSTVTSLSTYVFGTGTKLTVL

SEQ ID NO: 12 - protein, 247 aa, Artificial Sequence
  Synthetic_GUCY2C-binding scFv
EVQLVQSGAEVKRPGSSVKVSCKASGYTFTSYYMHWVRQAPGQGLEWMGIINPSGGSTSYAQKFQGRVTMTRDTSTSTVYMELSSLRSEDTAVYYCAAGTYSSGWTIDYWGQGTTVTVSSGGGGSGGGGSGGGASDIVMTQSPLSLPVTLGQPASISCRSSQSLVYTDGNTYLNWFQQRPGQSPRRLIYKVSNRDSGVPDRFSGSGSGTDFTLKISRVEAEDVGIYYCMHSKQWPPTFGGGTKVEIK

SEQ ID NO: 13 - protein, 238 aa, Artificial Sequence
  Synthetic_GUCY2C-binding scFv
EVQLVQSGAEVKKPGSSVKVSCKASGGTFSSYAISWVRQAPGQGLEWMGGIIPIFGTANYAQKFQGRVTITADKSTSTAYMELSSLRSEDTAVYYCARGHYYYMDVWGQGTTVTVSSGGGGSGGGGSGGGASDIVMTQSPATLSVSPGEGATLSCRASQSVSSNLAWYQQKPGRAPRLLIYGASTRATGIPARFSGSGSGTEFTLTISSLQSEDFAVYYCQQYNNWPSFGGGTKLEIK

SEQ ID NO: 14 - protein, 238 aa, Artificial Sequence
  Synthetic_GUCY2C-binding scFv
EVQLVQSGAEVKKPGSSVKVSCKASGGTFSSYAISWVRQAPGQGLEWMGGIIPIFGTANYAQKFQGRVTITADKSTSTAYMELSSLRSEDTAVYYCARGHYYYMDVWGQGTTVTVSSGGGGSGGGGSGGGASDIVMTQSPATLSVSPGEGATLSCRASQSVSSNLAWYQQKPGRAPRLLIYGASTRATGIPARFSGSGSGTEFTLTISSLQSEDFAVYYCQQYNNWPTFGGGTKLEIK

SEQ ID NO: 15 - protein, 247 aa, Artificial Sequence
  Synthetic_GUCY2C-binding scFv
QVQLVESGAEVKKPGSSVKVSCKASGGTFSSYAISWVRQAPGQGLEWMGGIIPIFGTANYAQKFQGRVTITADESTSTAYMELSGLRSEDTAVYYCARGIQPLRYYGMDVWGQGTLVTVSSGGGGSGGGGSGGGASQSALTQPPSASGTPGQRVTISCSGSSSNIGSNYVYWYQQLPGTAPKLLIYRNNQRPSGVPDRFSGSKSGTSASLAISGLRSEDEADYYCAAWDDSLSGRGVFGGGTQLTVL

SEQ ID NO: 16 - protein, 243 aa, Artificial Sequence
  Synthetic_GUCY2C-binding scFv
QVQLVESGGGLVKPGGSLRLSCAASGFTFSSYSMNWVRQAPGKGLEWVSVIYSGGSTHYADSVKGRFTISRHNSKNTLYLQMNSLRAEDTAVYYCARGAGTLNAFDIWGQGTTVTVSSGGGGSGGGGSGGGASQSGLTQPPSTSGSPGQSVTISCTGTSSDVGAYSYVSWYQQHPGKAPKLLIYAVTKRPSGVPDRFSGSKSGNTASLTVSGLQDEDEADYYCSSFAGGSTLVFGGGTKLTVL

SEQ ID NO: 17 - protein, 247 aa, Artificial Sequence
  Synthetic_GUCY2C-binding scFv
QMQLVQSGAEVKKPGSSVKVSCKASGGTFSSYAISWVRQAPGQGLEWMGGIIPIFGTANYAQKFQGRVTITADESTSTAYMELSSLRSEDTAVYYCVRGYSSIYYYYGMDVWGQGTMVTVSSGGGGSGGGGSGGGASQSGLTQPRSVSGSPGQSVTISCTGTSSDVGGYNYVSWYQQHPGKAPKLMIYDVSKRPSGVSDRFSGSKSGNTASLTISGLQAEDEADYYCGSYTSDGTLVFGGGTKLTVL

SEQ ID NO: 18 - protein, 243 aa, Artificial Sequence
  Synthetic_GUCY2C-binding scFv
QVQLVQSGAEVKKPGSSVKVSCKASGGTFSSYTISWVRQAPGQGLEWMGRIIPILGIANYAQKFQGRVTITADKSTSTAYMELSSLRSEDTAVYYCARDRSYNWLDPWGRGTLVTVSSGGGGSGGGGSGGGASQSALTQPVSVSGSPGQSITISCTGTISDVGDYNYVSWYQQHPGKAPKLMIYDVNNRPSGVSNRFSGSKSGNTASLTISGLQAEDEADYYCSSYTSSSTLVFGGGTKLTVL

SEQ ID NO: 19 - protein, 250 aa, Artificial Sequence
  Synthetic_GUCY2C-binding scFv
EIVMTQSPATLSVSPGERATLSCRASQSVSRNLAWYQQKPGQAPRLLIYGASTRATGIPARFSGSGSGTEFTLTIGSLQSEDFAVYYCQQYKTWPRTFGQGTNVEIKASGGGGSGGGGSGGGGSGGGGSELQVQLQQWGAGLLKPSETLSLTCAVFGGSFSGYYWSWIRQPPGKGLEWIGEINHRGNTNDNPSLKSRVTISVDTSKNQFALKLSSVTAADTAVYYCARERGYTYGNFDHWGQGTLVTVSS

SEQ ID NO: 20 - DNA, 738 bp, Artificial Sequence
  Synthetic_GUCY2C-binding scFv coding sequence
caggtgcagctggtgcagtctggggctgaggtgaagaagcctggggcctcagtgaaggtttcctgcaaggcatctggatacaccttcaccagctactatatgcactgggtgcgacaggcccctggacaagggcttgagtggatgggaataatcaaccctagtggtggtagcacaagctacgcacaggagttccagggcagagtcaccatgaccagggacacgtccacgagcacagtctacatggagctgagcagcctgagatctgaggacacggccgtgtattactgtgcgagagatgggcagtggcttcaatttgactactggggccaaggaaccctggtcaccgtctcgagtggtggaggcggttcaggcggaggtggctctggcggtggcgctagcgatattgtgatgacacagtctccactctccctgcccgtcacccttgggcagccggcctccatctcctgcaggtctagtcaaagcctcctaaaaaagagtgatgggaacacctacttgagttggtatcaccagaggccaggccaatctccacggcgcctaatttataaggtttctaatcgggactctggggtcccagacagattcagcggcagtgggtcagacactgatttcactctgaaaatcagcagagtggagactgaggatgttggaatttattactgcatgcaaggttcacactggcctccgacgttcggccaagggaccaaggtggaaatcaaa

SEQ ID NO: 21 - DNA, 729 bp, Artificial Sequence
  Synthetic_GUCY2C-binding scFv coding sequence
gaggtgcagctggtgcagcctggggctgaggtgaagaagcctgggtcctcggtgaaggtctcctgcaaggcttctggaggcaccctcagcagctatgctatcagctgggtgcgacaggcccctggacaagggcttgagtggatgggaaggatcatccctatccttggtataacaaactacgcacagaagttccagggcagagtcacgattaccgcggacaaatccacgagcacagcctacatggagctgagcagcctgagatctgaggacacggccgtgtatttctgtgcgagagatcagcggccggcgagcatggacgtctggggccagggcaccctggtcaccgtctcgagtggtggaggcggttcaggcggaggtggctctggcggtggcgctagccagtctgagctgactcagcctgcctccgtgtctgggtctcctggacagtcgatcaccatctcctgcactggaaccagcagtgacgttggtggttatatctatgtctcctggtaccaacagcacccaggcaaagtccccaaactcatgattcatgatgtcagtcatcggccctcaggggtttctaatcgcttctctggctccaggtctggcaacacggcctccctgaccatctctgggctccaggctgaggacgaggctgactatttctgcagctcatatgcaggcagcaacaattatgtcttcggaactgggaccaaggtcaccgtccta

SEQ ID NO: 22 - DNA, 735 bp, Artificial Sequence
  Synthetic_GUCY2C-binding scFv coding sequence
caggtccagctggtgcaatctggggctgaggtgaagaagcctgggtcctcggtgaaggtctcctgcaaggcttctggaggcaccttcagcagctatactatcagctgggtgcgacaggcccctggacaagagcttgagtggatgggaaggatcatccctatccttggtatagcaaactacgcacagaagttccagggcagagtcacgattaccgcggacaaatccacgagcacagcctacatggagctgagcagcctgagatctgaggacacggccgtgtattactgtgcgagagattatagcagcagctggaactctatggacgtctggggccagggaaccctggtcaccgtctcgagtggtggaggcggttcaggcggaggtggctctggcggtggcgctagccagtctgggctgactcagcctccctccgcgtccgggtctcctggacagtcagtcaccatctcctgcactggaaccagcagtgacattggttattatcactatgtctcctggtaccaacaacacccgggcaaagcccccaaactcatgatttatgaggacagtaagaggccctcagggatttctaatcgtttctctggctccaagtctggcaccacggcctccctgaccgtctctgggctccaggctgaggacgaggctcattattactgcagttcttttacaagtagaagtacttgggtgttcggcggagggacccagctcaccgtccta

SEQ ID NO: 23 - DNA, 729 bp, Artificial Sequence
  Synthetic_GUCY2C-binding scFv coding sequence
gaggtgcagctggtgcagcctggggctgaggtgaagaagcctgggtcctcggtgaaggtctcctgcaaggcttctggaggcaccctcagcagctatgctatcagctgggtgcgacaggcccctggacaagggcttgagtggatgggaaggatcatccctatccttggtataacaaactacgcacagaagttccagggcagagtcacgattaccgcggacaaatccacgagcacagcctacatggagctgagcagcctgagatctgaggacacggccgtgtatttctgtgcgagagatcagcggccggcgagcatggacgtctggggccagggcaccctggtcaccgtctcgagtggtggaggcggttcaggcggaggtggctctggcggtggcgctagccagtctgagctgactcagcctgcctccgtgtctgggtctcctggacagtcgatcaccatctcctgcactggaaccagcagtgacgttggtggttatatctatgtctcctggtaccaacagcacccaggcaaagtccccaaactcatgattcatgatgtcagtcatcggccctcaggggtttctaatcgcttctctggctccaggtctggcaacacggcctccctgaccatctctgggctccaggctgaggacgaggctgactatttctgcagctcatatacaagcagcaacaattattacttcggaactgggaccaaggtcaccgtccta

SEQ ID NO: 24 - DNA, 735 bp, Artificial Sequence
  Synthetic_GUCY2C-binding scFv coding sequence
caggtccagctggtgcaatctggggctgaggtgaagaagcctgggtcctcggtgaaggtctcctgcaaggcttctggaggcaccttcagcagctatactatcacctgggtgcgacaggcccctggacaagggcttgagtggatgggaaggatcatccctgtccttggtatagcaaactacgcacagaagttccagggcagagtcacgattaccgcggacaaatccacgagcacagcctacatggagctgagcagcctgagatctgaggacacggccgtgtattactgtgcgagagattatagcagcagctggaactctatggacgtctggggccagggaaccctggtcaccgtctcgagtggtggaggcggttcaggcggaggtggctctggcggtggcgctagccagtctgggctgactcagcctcgctcagtgtccgggtctcctggacagtcagtcaccatctcctgcactggaaccagcagtgatgttggtggttataactatgtctcctggtaccaacagcacccaggcaaagcccccaaactcatgatttatgatgtcagtaagcggccctcaggggtccctgatcgcttctccggctccaagtctgggaacacggcctccctgaccgtctctgggctccacgctgaggatgaggctgattattactgcagctcatatgcaggcagcaacaattttgtcttcggaactgggaccaaggtcaccgtccta

SEQ ID NO: 25 - DNA, 735 bp, Artificial Sequence
  Synthetic_GUCY2C-binding scFv coding sequence
caggtgcagctggtgcaatctggggctgaggtgaagaagcctgggtcctcggtgaaggtctcctgcaaggcttctggaggcaccttcggcagctatactatcagctgggtgcgacaggcccctggacaagggcttgagtggatgggaaggatcatccctatccttggtatagcaaactacgcacagaagttccagggcagagtcacgattaccgcggacaaatccacgagcacagcctacatggagctgagcagcctgagatctgaggacacggccgtgtattactgtgcgagagattatagcagcagctggaactctatggacgtctggggccaaggaaccctggtcaccgtctcgagtggtggaggcggttcaggcggaggtggctctggcggtggcgctagccagtctgggctgactcagcctcgctcagtgtccgggtctcctggacagtcagtcaccatctcctgcactggaaccagcagtgatgttggtgcttataactatgtctcctggtaccaacagcacccaggcaaagcccccaaactcatgatttatgaggtcagtaagcggccctcaggggtccctgatcgcttctctgcctccaagtctggcaacacggcctccctgaccgtctctgggctccaggctgaggatgaggctgattattactgcagctcatatgcaggcagcaacaattgggtgttcggcggagggaccaagctgaccgtccta

SEQ ID NO: 26 - DNA, 732 bp, Artificial Sequence
  Synthetic_GUCY2C-binding scFv coding sequence
caggtgcagctgcaggagtcgggcccagggcttgtgaagccttcggagaccctgtccctcacttgcactgtctctggtggctccatcagtagttactactggagctggatccggcagcccccagggaagggactggagtggattgggtctatctattacagtgggagcaccaactacaacccctccctcaagagtcgagtcaccatctcaagagacaagtcgaagaaccagttgtttctgaagttgaattctatgaccgccgcggacacggccgtctattattgtgcgagagatgtttggggcagtggccagtcatttgacagttggggccagggcaccctggtcaccgtctcgagtggtggaggcggttcaggcggaggtggctctggcggtggcgctagcaattttatgctgactcagccccactctgtgtcggagtctccggggaagacggtaaccatctcctgcacccgcagcagtggcagcattgccagcaactatgtgcagtggtaccagcagcgcttgggcagttcccccaccactgtgatctatgaacatagccgaagaccctctggggtccctgatcggttctctgcctccatcgacagctcctccaactctgcctccctcaccatctctggactgaagactgaggacgaggctgactactactgtcagtcttatgatgtcagcaatcgagtgttcggcggagggaccaagctgaccgtccta

SEQ ID NO: 27 - DNA, 738 bp, Artificial Sequence
  Synthetic_GUCY2C-binding scFv coding sequence
gaggtgcagctgttggagtctgggggaggcttggtccagcctggggggtccctgagactctcctgtgcagcctctggattcacctttagtagctattggatgagctgggtccgccaggctccagggaaggggctggagtgggtggccaacataaagcaagatggaagtgagaaatactatgtggactctgtgaagggccgattcaccatctccagagacaacgccaagaactcgctgtatctgcaaatgaacagcctgagagctgaggacacggctgtgtattattgtgcgaaagccccgtggtatagcagctcgccgacaccctacggtatggacgtctggggccagggcaccctggtcaccgtctcgagtggtggaggcggttcaggcggaggtggctctggcggtggcgctagcgacatccagatgacccagtctccatcctccctgtctgcatctgtaggagacagagtcaccatcacttgccaggcgagtcaggacattagcaactatttaaattggtatcagcagaaaccagggaaagcccctaggcgcctgatctatggtgcatccactttgatgagtggggtcccatcaaggttcagcggcagtggatctgggacagatttcactctcaccatcagcagtctgcaacctgaagattttgcaacttactactgtcaacagagttacagtacacctctcactttcggcggagggaccaaggtggaaatcaaa

SEQ ID NO: 28 - DNA, 738 bp, Artificial Sequence
  Synthetic_GUCY2C-binding scFv coding sequence
gaggtgcagctggtgcagtctggggctgaggtgaagaagcctgggtcctcggtgaaggtctcctgcaaggcttctggaggcaccttcagcagctatgctatcagctgggtgcgacaggcccctggacaagggcttgagtggatgggagggatcatccctatctttggtacagcaaactacgcacagaagttccagggcagagtcacgattaccgcggacgaatccacgagcacagcctacatggagctgagcagcctgagatctgaggacacggccgtgtattactgtgcgagaacacgttacatttgggggagttatcgggcatacggtatggacgtctggggccaagggacaatggtcaccgtctcgagtggtggaggcggttcaggcggaggtggctctggcggtggcgctagcgacatccagatgacccagtctccatcctccatgtctgcatctgtaggagacagagtcaccatcacttgccgcgcgagtcagagcattagcagtcatttaaattggtatcagcagctgccaggcaatgcccctactctcctgatctattatgcttccaatttacaaagtggggtcccatctaggttcagtggcagtggatctgggacagatttcactctcaccatcagcagtctgcagcctgatgattttgcaacttactactgtcaacagagtatcagtctcccgtacacttttggccaggggaccaaggtggagatcaaa

SEQ ID NO: 29 - DNA, 729 bp, Artificial Sequence
  Synthetic_GUCY2C-binding scFv coding sequence
gaggtgcagctggtgcagcctggggctgaggtgaagaagcctgggtcctcggtgaaggtctcctgcaaggcttctggaggcaccctcagcagctatgctatcagctgggtgcgacaggcccctggacaagggcttgagtggatgggaaggatcatccctatccttggtataacaaactacgcacagaagttccagggcagagtcacgattaccgcggacaaatccacgagcacagcctacatggagctgagcagcctgagatctgaggacacggccgtgtatttctgtgcgagagatcagcggccggcgagcatggacgtctggggccagggcaccctggtcaccgtctcgagtggtggaggcggttcaggcggaggtggctctggcggtggcgctagccagtctgagctgactcagcctgcctccgtgtctgggtctcctggacagtcgatcaccatctcctgcactggaaccagcagtgacgttggtggttatatctatgtctcctggtaccaacagcacccaggcaaagtccccaaactcatgattcatgatgtcagtcatcggccctcaggggtttctaatcgcttctctggctccaggtctggcaacacggcctccctgaccatctctgggctccaggctgaggacgaggctgactatttctgcagctcatatacaagcagcaacaattatgtcttcggaactgggaccaaggtcaccgtccta

SEQ ID NO: 30 - DNA, 729 bp, Artificial Sequence
  Synthetic_GUCY2C-binding scFv coding sequence
gaggtgcagctggtgcagcctggggctgaggtgaagaagcctgggtcctcggtgaaggtctcctgcaaggcttctggaggcaccctcagcagctatgctatcagctgggtgcgacaggcccctggacaagggcttgagtggatgggaaggatcatccctatccttggtataacaaactacgcacagaagttccagggcagagtcacgattaccgcggacaaatccacgagcacagcctacatggagctgagcagcctgagatctgaggacacggccgtgtatttctgtgcgagagatcagcggccggcgagcatggacgtctggggccagggcaccctggtcaccgtctcgagtggtggaggcggttcaggcggaggtggctctggcggtggcgctagccagtctgggctgactcagcctgcctccgtgtctgggtctcctggacagtcgatcaccatctcctgcactggaaccagcagtgatgttggtggttataactatgtctcctggtaccaacagcacccaggcaaagcccccaaactcatgatttatgaggtcagtaatcggccctcaggggtttctaatcgcttctctggctccaagtctggcaacacggcctccctgaccatctctgggctccaggctgaggacgaggctgattactactgcagcacagttacaagcctcagcacttatgtcttcggaactgggaccaagctgaccgtccta

SEQ ID NO: 31 - DNA, 741 bp, Artificial Sequence
  Synthetic_GUCY2C-binding scFv coding sequence
gaggtgcagctggtgcagtctggggctgaggtgaagaggcctgggtcctcggtgaaggtctcctgcaaggcatctggatacaccttcaccagctactatatgcactgggtgcgacaggcccctggacaagggcttgagtggatgggaataatcaaccctagtggtggtagcacaagctacgcacagaagttccagggcagagtcaccatgaccagggacacgtccacgagcacagtctacatggagctgagcagcctgagatctgaggacacggccgtgtattactgtgcggcaggaacgtatagcagtggctggacgattgactactgggggcaagggaccacggtcaccgtctcgagtggtggaggcggttcaggcggaggtggctctggcggtggcgctagcgatattgtgatgacgcagtctccactctccctgcccgtcacccttggacagccggcctccatctcctgcaggtctagtcaaagcctcgtatacactgatggaaacacctacttgaattggtttcagcagaggccaggccaatctccaaggcgcctaatttataaggtttctaaccgggactctggggtcccagacagattcagcggcagtgggtcaggcactgatttcacactgaaaatcagcagggtggaggctgaggatgttgggatttattactgcatgcatagtaaacagtggcctcccactttcggcggagggaccaaggtggaaatcaaa

SEQ ID NO: 32 - DNA, 714 bp, Artificial Sequence
  Synthetic_GUCY2C-binding scFv coding sequence
gaggtgcagctggtgcagtctggggctgaggtgaagaagcctgggtcctcggtgaaggtctcctgcaaggcttctggaggcaccttcagcagctatgctatcagctgggtgcgacaggcccctggacaagggcttgagtggatgggagggatcatccctatctttggtacagcaaactacgcacagaagttccagggcagagtcacgattaccgcggacaaatccacgagcacagcctacatggagctgagcagcctgagatctgaggacacggccgtgtattactgtgcgagaggacactactactacatggacgtctgggggcaagggaccacggtcaccgtctcgagtggtggaggcggttcaggcggaggtggctctggcggtggcgctagcgatattgtgatgactcagtctccagccaccctgtctgtgtctccaggggaaggagccaccctctcctgcagggccagtcagagtgttagcagcaacttagcctggtatcagcagaaacctggccgggctcccaggctcctcatctatggtgcatccaccagggccactggtatcccagccaggttcagtggcagtgggtctgggacagagttcactctcaccatcagcagcctgcagtctgaagattttgcagtttattactgtcagcagtataataactggcccagtttcggcggagggaccaagctggagatcaaa

SEQ ID NO: 33 - DNA, 714 bp, Artificial Sequence
  Synthetic_GUCY2C-binding scFv coding sequence
gaggtgcagctggtgcagtctggggctgaggtgaagaagcctgggtcctcggtgaaggtctcctgcaaggcttctggaggcaccttcagcagctatgctatcagctgggtgcgacaggcccctggacaagggcttgagtggatgggagggatcatccctatctttggtacagcaaactacgcacagaagttccagggcagagtcacgattaccgcggacaaatccacgagcacagcctacatggagctgagcagcctgagatctgaggacacggccgtgtattactgtgcgagaggacactactactacatggacgtctgggggcaagggaccacggtcaccgtctcgagtggtggaggcggttcaggcggaggtggctctggcggtggcgctagcgatattgtgatgactcagtctccagccaccctgtctgtgtctccaggggaaggagccaccctctcctgcagggccagtcagagtgttagcagcaacttagcctggtatcagcagaaacctggccgggctcccaggctcctcatctatggtgcatccaccagggccactggtatcccagccaggttcagtggcagtgggtctgggacagagttcactctcaccatcagcagcctgcagtctgaagattttgcagtttattactgtcagcagtataataactggcccactttcggcggagggaccaagctggagatcaaa

SEQ ID NO: 34 - DNA, 741 bp, Artificial Sequence
  Synthetic_GUCY2C-binding scFv coding sequence
caggtgcagctggtggagtctggggctgaggtgaagaagcctgggtcctcggtgaaggtctcctgcaaggcttctggaggcaccttcagcagctatgctatcagctgggtgcgacaggcccctggacaaggacttgagtggatgggagggatcatccctatctttggtacagcaaactacgcacagaagttccagggcagagtcacgattaccgcggacgaatccacgagcacagcctacatggagctgagcggcctgagatctgaggacacggccgtgtattactgtgcgagaggtatacagcctcttcgctactacggtatggacgtctggggccaaggaaccctggtcaccgtctcgagtggtggaggcggttcaggcggaggtggctctggcggtggcgctagccagtctgcgctgactcagccaccctcagcgtctgggacccccgggcagagggtcaccatctcttgttctggaagcagctccaacatcggaagtaattatgtatactggtaccagcagctcccaggaacggcccccaaactcctcatctataggaataatcagcggccctcaggggtccctgaccgattctctggctccaagtctggcacctcagcctccctggccatcagtgggctccggtccgaggatgaggctgattattactgtgcagcatgggatgacagcctgagtggtcggggagtgttcggcggagggacccagctcaccgtccta

SEQ ID NO: 35 - DNA, 729 bp, Artificial Sequence
  Synthetic_GUCY2C-binding scFv coding sequence
caggtgcagctggtggagtctgggggaggcctggtcaagcctggggggtccctgagactctcctgtgcagcctctggattcaccttcagtagctatagcatgaactgggtccgccaggctccagggaaggggctggagtgggtctcagttatttatagcggtggtagcacacactacgcagactccgtgaagggccgattcaccatctccagacacaattccaagaacacgctgtatcttcaaatgaacagcctgagagctgaggacacggccgtgtattactgtgcgaggggggctggtaccttaaatgcttttgatatctgggggcaagggaccacggtcaccgtctcgagtggtggaggcggttcaggcggaggtggctctggcggtggcgctagccagtctgggctgactcagcctccctccacgtccgggtctcctggacagtcagtcaccatctcctgcactggaaccagcagtgacgttggtgcttatagctatgtctcctggtatcaacaacacccaggcaaagcccccaaacttctcatttatgcggtcactaagaggccctcgggggtccctgatcgcttctctggctccaagtctggcaacacggcctccctgaccgtctctggactccaggatgaggatgaggctgattattactgcagctcttttgcaggcggcagcactctggtgttcggcggagggaccaagctgaccgtccta

SEQ ID NO: 36 - DNA, 741 bp, Artificial Sequence
  Synthetic_GUCY2C-binding scFv coding sequence
caaatgcagctggtgcagtctggggctgaggtgaagaagcctgggtcctcggtgaaggtctcctgcaaggcttctggaggcaccttcagcagctatgctatcagctgggtgcgacaggcccctggacaagggcttgagtggatgggagggatcatccctatctttggtacagcaaactatgcacagaagttccagggcagagtcacgattaccgcggacgaatccacgagcacagcctacatggagctgagcagcctgagatctgaggacacggccgtgtattactgtgtgagaggatacagttcaatatactactactacggtatggacgtctggggccaagggacaatggtcaccgtctcgagtggtggaggcggttcaggcggaggtggctctggcggtggcgctagccagtctgggctgactcagcctcgctcagtgtccgggtctcctggacagtcagtcaccatctcctgcactggaaccagcagtgatgttggtggttataactatgtctcctggtaccaacagcacccaggcaaagcccccaaactcatgatttatgatgtcagtaagcggccctcaggggtttctgatcgcttctctggctccaagtctggcaacacggcctccctgaccatctctgggctccaggctgaggacgaggctgattattactgcggctcatatacaagcgacgggactctagtattcggcggagggaccaagctgaccgtccta

SEQ ID NO: 37 - DNA, 729 bp, Artificial Sequence
  Synthetic_GUCY2C-binding scFv coding sequence
caggtgcagctggtgcaatctggggctgaggtgaagaagcctgggtcctcggtgaaggtctcctgcaaggcttctggaggcaccttcagcagctatactatcagctgggtgcgacaggcccctggacaagggcttgagtggatgggaaggatcatccctatccttggtatagcaaactacgcacagaagttccagggcagagtcacgattaccgcggacaaatccacgagcacagcctacatggagctgagcagcctgagatctgaggacacggccgtgtattactgtgcgagagataggtcttacaactggctcgacccctggggccgtggcaccctggtcaccgtctcgagtggtggaggcggttcaggcggaggtggctctggcggtggcgctagccagtctgcgctgactcagcctgtctccgtgtctgggtctcctggacagtcgatcaccatctcctgcactggaaccatcagtgacgttggtgattataactatgtctcctggtaccaacagcacccaggcaaagcccccaaactcatgatttatgacgtcaataatcggccctcaggggtttctaatcgcttctctggctccaagtctggcaacacggcctccctgaccatctctgggctccaggctgaggacgaggctgattattactgcagctcatatacaagcagcagcactctggtattcggcggagggaccaagctgaccgtccta

SEQ ID NO: 38 - protein, 8 aa, Artificial Sequence
  Synthetic_CDR-H1
GYTFTSYY

SEQ ID NO: 39 - protein, 8 aa, Artificial Sequence
  Synthetic_CDR-H1
GGTLSSYA

SEQ ID NO: 40 - protein, 8 aa, Artificial Sequence
  Synthetic_CDR-H1
GGTFSSYT

SEQ ID NO: 41 - protein, 8 aa, Artificial Sequence
  Synthetic_CDR-H1
GGTFGSYT

SEQ ID NO: 42 - protein, 8 aa, Artificial Sequence
  Synthetic_CDR-H1
GGSISSYY

SEQ ID NO: 43 - protein, 8 aa, Artificial Sequence
  Synthetic_CDR-H1
GFTFSSYW

SEQ ID NO: 44 - protein, 8 aa, Artificial Sequence
  Synthetic_CDR-H1
GGTFSSYA

SEQ ID NO: 45 - protein, 8 aa, Artificial Sequence
  Synthetic_CDR-H1
GFTFSSYS

SEQ ID NO: 46 - protein, 8 aa, Artificial Sequence
  Synthetic_CDR-H2
INPSGGST

SEQ ID NO: 47 - protein, 8 aa, Artificial Sequence
  Synthetic_CDR-H2
IIPILGIT

SEQ ID NO: 48 - protein, 8 aa, Artificial Sequence
  Synthetic_CDR-H2
IIPILGIA

SEQ ID NO: 49 - protein, 8 aa, Artificial Sequence
  Synthetic_CDR-H2
IIPVLGIA

SEQ ID NO: 50 - protein, 7 aa, Artificial Sequence
  Synthetic_CDR-H2
IYYSGST

SEQ ID NO: 51 - protein, 8 aa, Artificial Sequence
  Synthetic_CDR-H2
IKQDGSEK

SEQ ID NO: 52 - protein, 8 aa, Artificial Sequence
  Synthetic_CDR-H2
IIPIFGTA

SEQ ID NO: 53 - protein, 7 aa, Artificial Sequence
  Synthetic_CDR-H2
IYSGGST

SEQ ID NO: 54 - protein, 9 aa, Artificial Sequence
  Synthetic_CDR-H3
DGQWLQFDY

SEQ ID NO: 55 - protein, 9 aa, Artificial Sequence
  Synthetic_CDR-H3
DQRPASMDV

SEQ ID NO: 56 - protein, 11 aa, Artificial Sequence
  Synthetic_CDR-H3
DYSSSWNSMDV

SEQ ID NO: 57 - protein, 11 aa, Artificial Sequence
  Synthetic_CDR-H3
DVWGSGQSFDS

SEQ ID NO: 58 - protein, 15 aa, Artificial Sequence
  Synthetic_CDR-H3
APWYSSSPTPYGMDV

SEQ ID NO: 59 - protein, 15 aa, Artificial Sequence
  Synthetic_CDR-H3
TRYIWGSYRAYGMDV

SEQ ID NO: 60 - protein, 11 aa, Artificial Sequence
  Synthetic_CDR-H3
GTYSSGWTIDY

SEQ ID NO: 61 - protein, 8 aa, Artificial Sequence
  Synthetic_CDR-H3
GHYYYMDV

SEQ ID NO: 62 - protein, 12 aa, Artificial Sequence
  Synthetic_CDR-H3
GIQPLRYYGMDV

SEQ ID NO: 63 - protein, 10 aa, Artificial Sequence
  Synthetic_CDR-H3
GAGTLNAFDI

SEQ ID NO: 64 - protein, 13 aa, Artificial Sequence
  Synthetic_CDR-H3
GYSSIYYYYGMDV

SEQ ID NO: 65 - protein, 9 aa, Artificial Sequence
  Synthetic_CDR-H3
DRSYNWLDP

SEQ ID NO: 66 - protein, 12 aa, Artificial Sequence
  Synthetic_CDR-L1
QSLLKKSDGNTY

SEQ ID NO: 67 - protein, 9 aa, Artificial Sequence
  Synthetic_CDR-L1
SSDVGGYIY

SEQ ID NO: 68 - protein, 9 aa, Artificial Sequence
  Synthetic_CDR-L1
SSDIGYYHY

SEQ ID NO: 69 - protein, 9 aa, Artificial Sequence
  Synthetic_CDR-L1
SSDVGGYNY

SEQ ID NO: 70 - protein, 9 aa, Artificial Sequence
  Synthetic_CDR-L1
SSDVGAYNY

SEQ ID NO: 71 - protein, 8 aa, Artificial Sequence
  Synthetic_CDR-L1
SGSIASNY

SEQ ID NO: 72 - protein, 6 aa, Artificial Sequence
  Synthetic_CDR-L1
QDISNY

SEQ ID NO: 73 - protein, 6 aa, Artificial Sequence
  Synthetic_CDR-L1
QSISSH

SEQ ID NO: 74 - protein, 11 aa, Artificial Sequence
  Synthetic_CDR-L1
QSLVYTDGNTY

SEQ ID NO: 75 - protein, 6 aa, Artificial Sequence
  Synthetic_CDR-L1
QSVSSN

SEQ ID NO: 76 - protein, 8 aa, Artificial Sequence
  Synthetic_CDR-L1
SSNIGSNY

SEQ ID NO: 77 - protein, 9 aa, Artificial Sequence
  Synthetic_CDR-L1
SSDVGAYSY

SEQ ID NO: 78 - protein, 9 aa, Artificial Sequence
  Synthetic_CDR-L1
ISDVGDYNY

SEQ ID NO: 79 - protein, 3 aa, Artificial Sequence
  Synthetic_CDR-L2
KVS

SEQ ID NO: 80 - protein, 3 aa, Artificial Sequence
  Synthetic_CDR-L2
DVS

SEQ ID NO: 81 - protein, 3 aa, Artificial Sequence
  Synthetic_CDR-L2
EDS

SEQ ID NO: 82 - protein, 3 aa, Artificial Sequence
  Synthetic_CDR-L2
EVS

SEQ ID NO: 83 - protein, 3 aa, Artificial Sequence
  Synthetic_CDR-L2
EHS

SEQ ID NO: 84 - protein, 3 aa, Artificial Sequence
  Synthetic_CDR-L2
GAS

SEQ ID NO: 85 - protein, 3 aa, Artificial Sequence
  Synthetic_CDR-L2
YAS

SEQ ID NO: 86 - protein, 3 aa, Artificial Sequence
  Synthetic_CDR-L2
RNN

SEQ ID NO: 87 - protein, 3 aa, Artificial Sequence
  Synthetic_CDR-L2
AVT

SEQ ID NO: 88 - protein, 3 aa, Artificial Sequence
  Synthetic_CDR-L2
DVN

SEQ ID NO: 89 - protein, 9 aa, Artificial Sequence
  Synthetic_CDR-L3
MQGSHWPPT

SEQ ID NO: 90 - protein, 10 aa, Artificial Sequence
  Synthetic_CDR-L3
SSYAGSNNYV

SEQ ID NO: 91 - protein, 10 aa, Artificial Sequence
  Synthetic_CDR-L3
SSFTSRSTWV

SEQ ID NO: 92 - protein, 10 aa, Artificial Sequence
  Synthetic_CDR-L3
SSYTSSNNYY

SEQ ID NO: 93 - protein, 10 aa, Artificial Sequence
  Synthetic_CDR-L3
SSYAGSNNFV

SEQ ID NO: 94 - protein, 10 aa, Artificial Sequence
  Synthetic_CDR-L3
SSYAGSNNWV

SEQ ID NO: 95 - protein, 9 aa, Artificial Sequence
  Synthetic_CDR-L3
QSYDVSNRV

SEQ ID NO: 96 - protein, 9 aa, Artificial Sequence
  Synthetic_CDR-L3
QQSYSTPLT

SEQ ID NO: 97 - protein, 9 aa, Artificial Sequence
  Synthetic_CDR-L3
QQSISLPYT

SEQ ID NO: 98 - protein, 10 aa, Artificial Sequence
  Synthetic_CDR-L3
SSYTSSNNYV

SEQ ID NO: 99 - protein, 10 aa, Artificial Sequence
  Synthetic_CDR-L3
STVTSLSTYV

SEQ ID NO: 100 - protein, 9 aa, Artificial Sequence
  Synthetic_CDR-L3
MHSKQWPPT

SEQ ID NO: 101 - protein, 8 aa, Artificial Sequence
  Synthetic_CDR-L3
QQYNNWPS

SEQ ID NO: 102 - protein, 8 aa, Artificial Sequence
  Synthetic_CDR-L3
QQYNNWPT

SEQ ID NO: 103 - protein, 12 aa, Artificial Sequence
  Synthetic_CDR-L3
AAWDDSLSGRGV

SEQ ID NO: 104 - protein, 10 aa, Artificial Sequence
  Synthetic_CDR-L3
SSFAGGSTLV

SEQ ID NO: 105 - protein, 10 aa, Artificial Sequence
  Synthetic_CDR-L3
GSYTSDGTLV

SEQ ID NO: 106 - protein, 10 aa, Artificial Sequence
  Synthetic_CDR-L3
SSYTSSSTLV

SEQ ID NO: 107 - protein, 8 aa, Artificial Sequence
  Synthetic_CDR-H1
GGSFSGYY

SEQ ID NO: 108 - protein, 7 aa, Artificial Sequence
  Synthetic_CDR-H2
INHRGNT

SEQ ID NO: 109 - protein, 11 aa, Artificial Sequence
  Synthetic_CDR-H3
ERGYTYGNFDH

SEQ ID NO: 110 - protein, 6 aa, Artificial Sequence
  Synthetic_CDR-L1
QSVSRN

SEQ ID NO: 111 - protein, 9 aa, Artificial Sequence
  Synthetic_CDR-L3
QQYKTWPRT

SEQ ID NO: 112 - protein, 430 aa, Artificial Sequence
  Synthetic_Hu-GUCY2C
MKTLLLDLALWSLLFQPGWLSFSSQVSQNCHNGSYEISVLMMGNSAFAEPLKNLEDAVNEGLEIVRGRLQNAGLNVTVNATFMYSDGLIHNSGDCRSSTCEGLDLLRKISNAQRMGCVLIGPSCTYSTFQMYLDTELSYPMISAGSFGLSCDYKETLTRLMSPARKLMYFLVNFWKTNDLPFKTYSWSTSYVYKNGTETEDCFWYLNALEASVSYFSHELGFKVVLRQDKEFQDILMDHNRKSNVIIMCGGPEFLYKLKGDRAVAEDIVIILVDLFNDQYFEDNVTAPDYMKNVLVLTLSPGNSLLNSSFSRNLSPTKRDFALAYLNGILLFGHMLKIFLENGENITTPKFAHAFRNLTFEGYDGPVTLDDWGDVDSTMVLLYTSVDTKKYKVLLTYDTHVNKTYPVDMSPTFTWKNSKLPNDITGRGPQ

SEQ ID NO: 113 - protein, 430 aa, Artificial Sequence
  Synthetic_Mu-GUCY2C
MTSLLGLAVRLLLFQPALMVFWASQVRQNCRNGSYEISVLMMDNSAYKEPMQNLREAVEEGLDIVRKRLREADLNVTVNATFIYSDGLIHKSGDCRSSTCEGLDLLREITRDHKMGCALMGPSCTYSTFQMYLDTELNYPMISAGSYGLSCDYKETLTRILPPARKLMYFLVDFWKVNNASFKPFSWNSSYVYKNGSEPEDCFWYLNALEAGVSYFSEVLNFKDVLRRSEQFQEILTGHNRKSNVIVMCGTPESFYDVKGDLQVAEDTVVILVDLFSNHYFEENTTAPEYMDNVLVLTLPSEQSTSNTSVAERFSSGRSDFSLAYLEGTLLFGHMLQTFLENGENVTGPKFARAFRNLTFQGFAGPVTLDDSGDIDNIMSLLYVSLDTRKYKVLMKYDTHKNKTIPVAENPNFIWKNHKLPNDVPGLGPQ

SEQ ID NO: 114 - protein, 430 aa, Artificial Sequence
  Synthetic_Cy-GUCY2C
MKTLLLDLVLWSLLFQPEWLYLTSQVSQNCHNGSYEISVLMMDNSAFAEPLENVEDAVNEGLEIVRGRLQNAGLNVTVNASFMYSDGLIHNSGDCRSSTCEGLDLLRKISNAKRMGCVLMGPSCTYSTFQMYLDTELSYPMISAGSFGLSCDYKETLTRLMSPARKLTYFLVNFWKTNDLPFKTYSWSTSYVYKNGTESEDCFWYLNALEASVSYFSHELSFKLVLRQDKEFQDILMDHNRKSNVIVMCGDPQFLYKLKGDRAVAEDIVIILVDLFNDQYFEDNVTAPDYMKNVLVLTQSPGNSLLNSSFSRNLSPTKRDFALAYLNGILLFGHMLKTFLENGENITTPKFAHAFRNLTFEGYDGPVTLDDWGDVDSTMVLLYTSVDTKKYKVLLTYDTHVNQTNPVDMSPTFTWKNSKLPNDITDRGPQ

SEQ ID NO: 115 - protein, 182 aa, Artificial Sequence
  Synthetic_rCD4
TSITAYKSEGESAEFSFPLNLGEESLQGELRWKAEKAPSSQSWITFSLKNQKVSVQKSTSNPKFQLSETLPLTLQIPQVSLQFAGSGNLTLTLDRGILYQEVNLVVMKVTQPDSNTLTCEVMGPTSPKMRLILKQENQEARVSRQEKVIQVQAPEAGVWQCLLSEGEEVKMDSKIQVLSKGL